European Patent Application EP 4 760 258 A2, published June 17, 2026. Title: Therapy Guidance and/or Therapy Monitoring for a treatment with Angiotensin-Receptor-Agonist and/or a Precursor thereof. Applicant: 4Teen4 Pharmaceuticals GmbH. Application EP, filed December 20, 2019. The sequence listing filed with the application follows.

SEQUENCE LISTING (47 sequences)

SEQ ID NO: 1 - protein, 737 aa, Homo sapiens
MADTQYILPNDIGVSSLDCREAFRLLSPTERLYAYHLSRAAWYGGLAVLLQTSPEAPYIYALLSRLFRAQDPDQLRQHALAEGLTEEEYQAFLVYAAGVYSNMGNYKSFGDTKFVPNLPKEKLERVILGSEAAQQHPEEVRGLWQTCGELMFSLEPRLRHLGLGKEGITTYFSGNCTMEDAKLAQDFLDSQNLSAYNTRLFKEVDGEGKPYYEVRLASVLGSEPSLDSEVTSKLKSYEFRGSPFQVTRGDYAPILQKVVEQLEKAKAYAANSHQGQMLAQYIESFTQGSIEAHKRGSRFWIQDKGPIVESYIGFIESYRDPFGSRGEFEGFVAVVNKAMSAKFERLVASAEQLLKELPWPPTFEKDKFLTPDFTSLDVLTFAGSGIPAGINIPNYDDLRQTEGFKNVSLGNVLAVAYATQREKLTFLEEDDKDLYILWKGPSFDVQVGLHELLGHGSGKLFVQDEKGAFNFDQETVINPETGEQIQSWYRSGETWDSKFSTIASSYEECRAESVGLYLCLHPQVLEIFGFEGADAEDVIYVNWLNMVRAGLLALEFYTPEAFNWRQAHMQARFVILRVLLEAGEGLVTITPTTGSDGRPDARVRLDRSKIRSVGKPALERFLRRLQVLKSTGDVAGGRALYEGYATVTDAPPECFLTLRDTVLLRKESRKLIVQPNTRLEGSDVQLLEYEASAAGLIRSFSERFPEDGPELEEILTQLATADARFWKGPSEAPSGQA

SEQ ID NO: 2 - protein, 21 aa, Homo sapiens
CETVINPETGEQIQSWYRSGE

SEQ ID NO: 3 - protein, 6 aa, Homo sapiens
INPETG

SEQ ID NO: 4 - protein, 116 aa, Mus musculus
QVTLKESGPGILQPSQTLSLTCSFSGFSLSTSGMSVGWIRQPSGKGLEWLAHIWWNDNKSYNPALKSRLTISRDTSNNQVFLKIASVVTADTGTYFCARNYSYDYWGQGTTLTVSS

SEQ ID NO: 5 - protein, 112 aa, Mus musculus
DVVVTQTPLSLSVSLGDPASISCRSSRSLVHSIGSTYLHWYLQKPGQSPKLLIYKVSNRFSGVPDRFSGSGSGTDFTLKISRVEAEDLGVYFCSQSTHVPWTFGGGTKLEIK

SEQ ID NO: 6 - protein, 10 aa, Mus musculus
GFSLSTSGMS

SEQ ID NO: 7 - protein, 7 aa, Mus musculus
IWWNDNK

SEQ ID NO: 8 - protein, 8 aa, Mus musculus
ARNYSYDY

SEQ ID NO: 9 - protein, 11 aa, Mus musculus
RSLVHSIGSTY

SEQ ID NO: 10 - protein, 9 aa, Mus musculus
SQSTHVPWT

SEQ ID NO: 11 - protein, 469 aa, Homo sapiens
MDPKGSLSWRILLFLSLAFELSYGQITLKESGPTLVKPTQTLTLTCTFSGFSLSTSGMSVGWIRQPPGKALEWLAHIWWNDNKSYNPALKSRLTITRDTSKNQVVLTMTNMDPVDTGTYYCARNYSYDYWGQGTLVTVSSASTKGPSVFPLAPSSKSTSGGTAALGCLVKDYFPEPVTVSWNSGALTSGVHTFPAVLQSSGLYSLSSVVTVPSSSLGTQTYICNVNHKPSNTKVDKKVEPKSCDKTHTCPPCPAPELLGGPSVFLFPPKPKDTLMISRTPEVTCVVVDVSHEDPEVKFNWYVDGVEVHNAKTKPREEQYNSTYRVVSVLTVLHQDWLNGKEYKCKVSNKALPAPIEKTISKAKGQPREPQVYTLPPSRDELTKNQVSLTCLVKGFYPSDIAVEWESNGQPENNYKTTPPVLDSDGSFFLYSKLTVDKSRWQQGNVFSCSVMHEALHNHYTQKSLSLSPG

SEQ ID NO: 12 - protein, 239 aa, Homo sapiens
METDTLLLWVLLLWVPGSTGDIVMTQTPLSLSVTPGQPASISCKSSRSLVHSIGSTYLYWYLQKPGQSPQLLIYKVSNRFSGVPDRFSGSGSGTDFTLKISRVEAEDVGVYYCSQSTHVPWTFGGGTKVEIKRTVAAPSVFIFPPSDEQLKSGTASVVCLLNNFYPREAKVQWKVDNALQSGNSQESVTEQDSKDSTYSLSSTLTLSKADYEKHKVYACEVTHQGLSSPVTKSFNRGEC

SEQ ID NO: 13 - protein, 8 aa, Homo sapiens
DRVYIHPF

SEQ ID NO: 14 - protein, 8 aa, synthetic construct
  REGION 1..8: note = Angiotensin II variant
DRVYVHPF

SEQ ID NO: 15 - protein, 8 aa, synthetic construct
  REGION 1..8: note = Angiotensin II variant
NRVFIHPF

SEQ ID NO: 16 - protein, 6 aa, Homo sapiens
VYIHPF

SEQ ID NO: 17 - protein, 9 aa, Homo sapiens
NRVYYVHPF

SEQ ID NO: 18 - protein, 8 aa, synthetic construct
  REGION 1..8: note = Angiotensin II analogue
NRVYIHPI

SEQ ID NO: 19 - protein, 8 aa, synthetic construct
  REGION 1..8: note = Angiotensin II analogue
NRVYIHPA

SEQ ID NO: 20 - protein, 8 aa, synthetic construct
  REGION 1..8: note = Angiotensin II analogue
NRVYIHPF

SEQ ID NO: 21 - protein, 7 aa, Homo sapiens
RVYIHPF

SEQ ID NO: 22 - protein, 7 aa, synthetic construct
  REGION 1..7: note = Angiotensin III analogue
RVYVHPF

SEQ ID NO: 23 - protein, 7 aa, synthetic construct
  REGION 1..7: note = Angiotensin III analogue
RVFIHPF

SEQ ID NO: 24 - protein, 7 aa, synthetic construct
  REGION 1..7: note = Angiotensin III analogue
RVYIHPA

SEQ ID NO: 25 - protein, 7 aa, synthetic construct
  REGION 1..7: note = Angiotensin III analogue
RVYIHPF

SEQ ID NO: 26 - protein, 6 aa, Homo sapiens
VYIHPF

SEQ ID NO: 27 - protein, 6 aa, synthetic construct
  REGION 1..6: note = Angiotensin IV analogue
VYVHPF

SEQ ID NO: 28 - protein, 6 aa, synthetic construct
  REGION 1..6: note = Angiotensin IV analogue
VFIHPF

SEQ ID NO: 29 - protein, 6 aa, synthetic construct
  REGION 1..6: note = Angiotensing IV analogue
VYIHPA

SEQ ID NO: 30 - protein, 6 aa, synthetic construct
  REGION 1..6: note = Angiotensin IV analogue
VYIHPF

SEQ ID NO: 31 - protein, 25 aa, synthetic construct
  MOD_RES 1: note = N-terminal biotinylation
AFNFDQETVINPETGEQIQSWYRSG

SEQ ID NO: 32 - protein, 19 aa, synthetic construct
  MOD_RES 1: note = N-terminal biotinylation
AFNFDQETVINPETGEQIQ

SEQ ID NO: 33 - protein, 18 aa, synthetic construct
  MOD_RES 1: note = N-terminal biotinylation
AFNFDQETVINPETGEQI

SEQ ID NO: 34 - protein, 17 aa, synthetic construct
  MOD_RES 1: note = N-terminal biotinylation
AFNFDQETVINPETGEQ

SEQ ID NO: 35 - protein, 16 aa, synthetic construct
  MOD_RES 1: note = N-terminal biotinylation
AFNFDQETVINPETGE

SEQ ID NO: 36 - protein, 15 aa, synthetic construct
  MOD_RES 1: note = N-terminal biotinylation
AFNFDQETVINPETG

SEQ ID NO: 37 - protein, 14 aa, synthetic construct
  MOD_RES 1: note = N-terminal biotinylation
AFNFDQETVINPET

SEQ ID NO: 38 - protein, 13 aa, synthetic construct
  MOD_RES 1: note = N-terminal biotinylation
AFNFDQETVINPE

SEQ ID NO: 39 - protein, 12 aa, synthetic construct
  MOD_RES 1: note = N-terminal biotinylation
AFNFDQETVINP

SEQ ID NO: 40 - protein, 11 aa, synthetic construct
  MOD_RES 1: note = N-terminal biotinylation
AFNFDQETVIN

SEQ ID NO: 41 - protein, 11 aa, synthetic construct
  MOD_RES 11: note = C-terminal biotinylation
ETGEQIQSWYK

SEQ ID NO: 42 - protein, 12 aa, synthetic construct
  MOD_RES 12: note = C-terminal biotinylation
PETGEQIQSWYK

SEQ ID NO: 43 - protein, 13 aa, synthetic construct
  MOD_RES 13: note = C-terminal biotinylation
NPETGEQIQSWYK

SEQ ID NO: 44 - protein, 14 aa, synthetic construct
  MOD_RES 14: note = C-terminal biotinylation
INPETGEQIQSWYK

SEQ ID NO: 45 - protein, 15 aa, synthetic construct
  MOD_RES 15: note = C-terminal biotinylation
VINPETGEQIQSWYK

SEQ ID NO: 46 - protein, 16 aa, synthetic construct
  MOD_RES 16: note = C-terminal biotinylation
TVINPETGEQIQSWYK

SEQ ID NO: 47 - protein, 17 aa, synthetic construct
  MOD_RES 17: note = C-terminal biotinylation
ETVINPETGEQIQSWYK